European Patent Application EP 4 356 927 A2, published April 24, 2024. Title: ANTIBODY BASED REAGENTS THAT SPECIFICALLY RECOGNIZE TOXIC OLIGOMERIC FORMS OF TAU. Applicant: ARIZONA BOARD OF REGENTS, A BODY CORPORATE OF THE STATE OF ARIZONA, ACTING FOR AND ON BEHALF OF ARIZONA STATE UNIVERSITY. The sequence listing filed with the application follows.

SEQUENCE LISTING (50 sequences)

SEQ ID NO: 1 - protein, 300 aa, synthetic construct
  REGION 1..300: note = Description of Artificial Sequence: Synthetic polypeptide
  MOD_RES 1: note = Any amino acid
  MOD_RES 3: note = Any amino acid
  MOD_RES 297..300: note = Any amino acid
XEXVIMKYLLPTAAAGLLLLAAQPAMAQVQLQESGGGVVQPGRSLRLSCAASGFTFSTSGMHWVRQAPGKGLEWVAFILHDGSDKYYADSVKGRFTISRDNSKNTLYLQMNSLRAEDTAIYYCAKSQRELLGAEYLQNWGQGTLVTVSSGGGGSGGGGSGGGGSQSALTQPASVSGSPGQSITISCTGTSSDVGGYKYVSWYQQHPGKAPKVMIYDVSNRPSGVSNRFSGSKSGNTASLTISGLQAEDEADYYCSSYTSSSTLVFGGGTKVTVLGAAAHHHHHHGAAEQKLISEEDXXXX

SEQ ID NO: 2 - DNA, 991 bp, synthetic construct
  misc_feature 1..991: note = Description of Artificial Sequence: Synthetic polynucleotide
  modified_base 12: mod_base = OTHER; note = a, c, t, g, unknown or other
  modified_base 888: mod_base = OTHER; note = a, c, t, g, unknown or other
  modified_base 902: mod_base = OTHER; note = a, c, t, g, unknown or other
  modified_base 907: mod_base = OTHER; note = a, c, t, g, unknown or other
  modified_base 911..913: mod_base = OTHER; note = a, c, t, g, unknown or other
  modified_base 920..921: mod_base = OTHER; note = a, c, t, g, unknown or other
  modified_base 945: mod_base = OTHER; note = a, c, t, g, unknown or other
  modified_base 948: mod_base = OTHER; note = a, c, t, g, unknown or other
  modified_base 951: mod_base = OTHER; note = a, c, t, g, unknown or other
  modified_base 962..963: mod_base = OTHER; note = a, c, t, g, unknown or other
  modified_base 971: mod_base = OTHER; note = a, c, t, g, unknown or other
  modified_base 977: mod_base = OTHER; note = a, c, t, g, unknown or other
  modified_base 979..983: mod_base = OTHER; note = a, c, t, g, unknown or other
  modified_base 989: mod_base = OTHER; note = a, c, t, g, unknown or other
  source 1..991: mol_type = other DNA
aattctatttcnggagacagtcataatgaaatacctattgcctacggcagccgctggattgttattactcgcggcccagccggccatggcccaggtgcagctgcaggagtcgggggaggcgtggtccagcctgggaggtccctgagactctcctgtgcagcgtctggattcaccttcagtacttctggcatgcactgggtccgccaggctccaggcaaggggctggagtgggtggcatttatactacatgatggaagtgataaatactatgcagactccgtgaagggccgattcaccatctccagagacaattccaagaacacgctgtatctgcaaatgaacagcctgagagccgaggacacggccatatattactgtgcgaaatctcagagggagctactcggcgctgaatacctccagaactggggccagggcaccctggtcaccgtctcctcaggtggaggcggttcaggcggaggtggctctggcggtggcggatcgcagtctgctctgactcagcctgcctccgtgtctgggtctcctggacagtcgatcaccatctcctgcactggaaccagcagtgacgttggtggttataagtatgtctcctggtaccaacagcacccaggcaaagcccccaaagtcatgatttatgatgtcagtaatcggccctcaggggtttctaatcgcttctctggctccaagtctggcaacacggcctccctgaccatctctgggctccaggctgaggacgaggctgattattactgcagctcatatacaagcagcagcactctcgtgttcggcggcgggaccaaggtcaccgtcctaggtgcggccgcagaacaaaaactcatctcagaagaggatctgaatggggccgcatanactgttgaaagttntttancaannntcatacnnaaaattcatttactaacgtctggnaanacnacaaaactttnnatcgttangctaantnnnnnagggcngt

SEQ ID NO: 3 - DNA, 902 bp, synthetic construct
  misc_feature 1..902: note = Description of Artificial Sequence: Synthetic polynucleotide
  modified_base 4..5: mod_base = OTHER; note = a, c, t, g, unknown or other
  modified_base 10: mod_base = OTHER; note = a, c, t, g, unknown or other
  modified_base 892..893: mod_base = OTHER; note = a, c, t, g, unknown or other
  modified_base 896..900: mod_base = OTHER; note = a, c, t, g, unknown or other
  source 1..902: mol_type = other DNA
ttcnngaganagtcataatgaaatacctattgcctacggcagccgctggattgttattactcgcggcccagccggccatggcccaggtgcagctgcaggagtctgggggaggcgtggtccagcctgggaggtccctgagactctcctgtgcagcgtctggattcaccttcagtacttctggcatgcactgggtccgccaggctccaggcaaggggctggagtgggtggcatttatactacatgatggaagtgataaatactatgcagactccgtgaagggccgattcaccatctccagagacaattccaagaacacgctgtatctgcaaatgaacagcctgagagccgaggacacggccatatattactgtgcgaaatctcagagggagctactcggcgctgaatacctccagaactggggccagggcaccctggtcaccgtctcctcaggtggaggcggttcaggcggaggtggctctggcggtggcggatcgcagtctgctctgactcagcctgcctccgtgtctgggtctcctggacagtcgatcaccatctcctgcactggaaccagcagtgacgttggtggttataagtatgtctcctggtaccaacagcacccaggcaaagcccccaaagtcatgatttatgatgtcagtaatcggccctcaggggtttctaatcgcttctctggctccaagtctggcaacacggcctccctgaccatctctgggctccaggctgaggacgaggctgattattactgcagctcatatacaagcagcagcactctcgtgttcggcggcgggaccaaggtcaccgtcctaggtgcggccgcacatcatcatcaccatcacggggccgcagaacaaaaactcatctcagaagaggatcnnaannnnncg

SEQ ID NO: 4 - DNA, 902 bp, synthetic construct; identical to SEQ ID NO: 3
  misc_feature 1..902: note = Description of Artificial Sequence: Synthetic polynucleotide
  modified_base 4..5: mod_base = OTHER; note = a, c, t, g, unknown or other
  modified_base 10: mod_base = OTHER; note = a, c, t, g, unknown or other
  modified_base 892..893: mod_base = OTHER; note = a, c, t, g, unknown or other
  modified_base 896..900: mod_base = OTHER; note = a, c, t, g, unknown or other
  source 1..902: mol_type = other DNA

SEQ ID NO: 5 - DNA, 991 bp, synthetic construct; identical to SEQ ID NO: 2
  misc_feature 1..991: note = Description of Artificial Sequence: Synthetic polynucleotide
  modified_base 12: mod_base = OTHER; note = a, c, t, g, unknown or other
  modified_base 888: mod_base = OTHER; note = a, c, t, g, unknown or other
  modified_base 902: mod_base = OTHER; note = a, c, t, g, unknown or other
  modified_base 907: mod_base = OTHER; note = a, c, t, g, unknown or other
  modified_base 911..913: mod_base = OTHER; note = a, c, t, g, unknown or other
  modified_base 920..921: mod_base = OTHER; note = a, c, t, g, unknown or other
  modified_base 945: mod_base = OTHER; note = a, c, t, g, unknown or other
  modified_base 948: mod_base = OTHER; note = a, c, t, g, unknown or other
  modified_base 951: mod_base = OTHER; note = a, c, t, g, unknown or other
  modified_base 962..963: mod_base = OTHER; note = a, c, t, g, unknown or other
  modified_base 971: mod_base = OTHER; note = a, c, t, g, unknown or other
  modified_base 977: mod_base = OTHER; note = a, c, t, g, unknown or other
  modified_base 979..983: mod_base = OTHER; note = a, c, t, g, unknown or other
  modified_base 989: mod_base = OTHER; note = a, c, t, g, unknown or other
  source 1..991: mol_type = other DNA

SEQ ID NO: 6 - DNA, 1002 bp, synthetic construct
  misc_feature 1..1002: note = Description of Artificial Sequence: Synthetic polynucleotide
  modified_base 4..5: mod_base = OTHER; note = a, c, t, g, unknown or other
  modified_base 10: mod_base = OTHER; note = a, c, t, g, unknown or other
  modified_base 743: mod_base = OTHER; note = a, c, t, g, unknown or other
  modified_base 799..800: mod_base = OTHER; note = a, c, t, g, unknown or other
  modified_base 824..826: mod_base = OTHER; note = a, c, t, g, unknown or other
  modified_base 862: mod_base = OTHER; note = a, c, t, g, unknown or other
  modified_base 878..879: mod_base = OTHER; note = a, c, t, g, unknown or other
  modified_base 881: mod_base = OTHER; note = a, c, t, g, unknown or other
  modified_base 900: mod_base = OTHER; note = a, c, t, g, unknown or other
  modified_base 903: mod_base = OTHER; note = a, c, t, g, unknown or other
  modified_base 908: mod_base = OTHER; note = a, c, t, g, unknown or other
  modified_base 921: mod_base = OTHER; note = a, c, t, g, unknown or other
  modified_base 931: mod_base = OTHER; note = a, c, t, g, unknown or other
  modified_base 935..936: mod_base = OTHER; note = a, c, t, g, unknown or other
  modified_base 965..969: mod_base = OTHER; note = a, c, t, g, unknown or other
  modified_base 977: mod_base = OTHER; note = a, c, t, g, unknown or other
  modified_base 980: mod_base = OTHER; note = a, c, t, g, unknown or other
  modified_base 985..988: mod_base = OTHER; note = a, c, t, g, unknown or other
  modified_base 992: mod_base = OTHER; note = a, c, t, g, unknown or other
  modified_base 996..1000: mod_base = OTHER; note = a, c, t, g, unknown or other
  modified_base 1002: mod_base = OTHER; note = a, c, t, g, unknown or other
  source 1..1002: mol_type = other DNA
ttcnngaganagtcataatgaaatacctattgcctacggcagccgctggattgttattactcgcggcccagccggccatggcccaggtgcagctgcaggagtctgggggaggcgtggtccagcctgggaggtccctgagactctcctgtgcagcgtctggattcaccttcagtacttctggcatgcactgggtccgccaggctccaggcaaggggctggagtgggtggcatttatactacatgatggaagtgataaatactatgcagactccgtgaagggccgattcaccatctccagagacaattccaagaacacgctgtatctgcaaatgaacagcctgagagccgaggacacggccatatattactgtgcgaaatctcagagggagctactcggcgctgaatacctccagaactggggccagggcaccctggtcaccgtctcctcaggtggaggcggttcaggcggaggtggctctggcggtggcggatcgcagtctgctctgactcagcctgcctccgtgtctgggtctcctggacagtcgatcaccatctcctgcactggaaccagcagtgacgttggtggttataagtatgtctcctggtaccaacagcacccaggcaaagcccccaaagtcatgatttatgatgtcagtaatcggccctcaggggtttctaatcgcttctctggctccaagtctggcaacacggcctccctgaccatctctgggctccaggctgangacgaggctgattattactgcagctcatatacaagcagcagcactctcgtgttcgnnggcgggaccaaggtcaccgtcctnnngcggccgcacatcatcatcaccatcacggggccgcngacaaaactcatctcnnanaggatctgaatgggccgcntanactgntgaaagttgttancaaaacctcntacnnaaaattcatttactaacgtctggaaagannnnnaactttanatngttannnnaacnatgnnnnngn

SEQ ID NO: 7 - DNA, 991 bp, synthetic construct
  misc_feature 1..991: note = Description of Artificial Sequence: Synthetic polynucleotide
  modified_base 2..6: mod_base = OTHER; note = a, c, t, g, unknown or other
  modified_base 8..11: mod_base = OTHER; note = a, c, t, g, unknown or other
  modified_base 16: mod_base = OTHER; note = a, c, t, g, unknown or other
  modified_base 19: mod_base = OTHER; note = a, c, t, g, unknown or other
  modified_base 24..29: mod_base = OTHER; note = a, c, t, g, unknown or other
  modified_base 35..36: mod_base = OTHER; note = a, c, t, g, unknown or other
  modified_base 38: mod_base = OTHER; note = a, c, t, g, unknown or other
  modified_base 58: mod_base = OTHER; note = a, c, t, g, unknown or other
  modified_base 85: mod_base = OTHER; note = a, c, t, g, unknown or other
  modified_base 116: mod_base = OTHER; note = a, c, t, g, unknown or other
  modified_base 123: mod_base = OTHER; note = a, c, t, g, unknown or other
  modified_base 127..129: mod_base = OTHER; note = a, c, t, g, unknown or other
  modified_base 132..133: mod_base = OTHER; note = a, c, t, g, unknown or other
  modified_base 135..137: mod_base = OTHER; note = a, c, t, g, unknown or other
  modified_base 142..143: mod_base = OTHER; note = a, c, t, g, unknown or other
  modified_base 206: mod_base = OTHER; note = a, c, t, g, unknown or other
  modified_base 222: mod_base = OTHER; note = a, c, t, g, unknown or other
  modified_base 224..225: mod_base = OTHER; note = a, c, t, g, unknown or other
  modified_base 981..982: mod_base = OTHER; note = a, c, t, g, unknown or other
  modified_base 985..989: mod_base = OTHER; note = a, c, t, g, unknown or other
  source 1..991: mol_type = other DNA
gnnnnntnnnnggaantgngagcnnnnnnaatttnncncaggaaacagctatgaccangattacgccaagcttgcatgcaaattntatttcaaggagacagtcataatgaaatacntattgcntacnnncanncnnnggatnntattactcgcggcccagccggccatggcccaggtgcagctgcaggagtctgggggaggcgtgntccagcctgggaggtncnngagactctcctgtgcagcgtctggattcaccttcagtacttctggcatgcactgggtccgccaggctccaggcaaggggctggagtgggtggcatttatactacatgatggaagtgataaatactatgcagactccgtgaagggccgattcaccatctccagagacaattccaagaacacgctgtatctgcaaatgaacagcctgagagccgaggacacggccatatattactgtgcgaaatctcagagggagctactcggcgctgaatacctccagaactggggccagggcaccctggtcaccgtctcctcaggtggaggcggttcaggcggaggtggctctggcggtggcggatcgcagtctgctctgactcagcctgcctccgtgtctgggtctcctggacagtcgatcaccatctcctgcactggaaccagcagtgacgttggtggttataagtatgtctcctggtaccaacagcacccaggcaaagcccccaaagtcatgatttatgatgtcagtaatcggccctcaggggtttctaatcgcttctctggctccaagtctggcaacacggcctccctgaccatctctgggctccaggctgaggacgaggctgattattactgcagctcatatacaagcagcagcactctcgtgttcggcggcgggaccaaggtcaccgtcctaggtgcggccgcacatcatcatcaccatcacggggccgcagaacaaaaactcatctcagaagaggatcnnaannnnncg

SEQ ID NO: 8 - DNA, 992 bp, synthetic construct
  misc_feature 1..992: note = Description of Artificial Sequence: Synthetic polynucleotide
  modified_base 12: mod_base = OTHER; note = a, c, t, g, unknown or other
  modified_base 889: mod_base = OTHER; note = a, c, t, g, unknown or other
  modified_base 903: mod_base = OTHER; note = a, c, t, g, unknown or other
  modified_base 908: mod_base = OTHER; note = a, c, t, g, unknown or other
  modified_base 912..914: mod_base = OTHER; note = a, c, t, g, unknown or other
  modified_base 921..922: mod_base = OTHER; note = a, c, t, g, unknown or other
  modified_base 946: mod_base = OTHER; note = a, c, t, g, unknown or other
  modified_base 949: mod_base = OTHER; note = a, c, t, g, unknown or other
  modified_base 952: mod_base = OTHER; note = a, c, t, g, unknown or other
  modified_base 963..964: mod_base = OTHER; note = a, c, t, g, unknown or other
  modified_base 972: mod_base = OTHER; note = a, c, t, g, unknown or other
  modified_base 978: mod_base = OTHER; note = a, c, t, g, unknown or other
  modified_base 980..984: mod_base = OTHER; note = a, c, t, g, unknown or other
  modified_base 990: mod_base = OTHER; note = a, c, t, g, unknown or other
  source 1..992: mol_type = other DNA
aattctatttcnggagacagtcataatgaaatacctattgcctacggcagccgctggattgttattactcgcggcccagccggccatggcccaggtgcagctgcaggagtctgggggaggcgtggtccagcctgggaggtccctgagactctcctgtgcagcgtctggattcaccttcagtacttctggcatgcactgggtccgccaggctccaggcaaggggctggagtgggtggcatttatactacatgatggaagtgataaatactatgcagactccgtgaagggccgattcaccatctccagagacaattccaagaacacgctgtatctgcaaatgaacagcctgagagccgaggacacggccatatattactgtgcgaaatctcagagggagctactcggcgctgaatacctccagaactggggccagggcaccctggtcaccgtctcctcaggtggaggcggttcaggcggaggtggctctggcggtggcggatcgcagtctgctctgactcagcctgcctccgtgtctgggtctcctggacagtcgatcaccatctcctgcactggaaccagcagtgacgttggtggttataagtatgtctcctggtaccaacagcacccaggcaaagcccccaaagtcatgatttatgatgtcagtaatcggccctcaggggtttctaatcgcttctctggctccaagtctggcaacacggcctccctgaccatctctgggctccaggctgaggacgaggctgattattactgcagctcatatacaagcagcagcactctcgtgttcggcggcgggaccaaggtcaccgtcctaggtgcggccgcagaacaaaaactcatctcagaagaggatctgaatggggccgcatanactgttgaaagttntttancaannntcatacnnaaaattcatttactaacgtctggnaanacnacaaaactttnnatcgttangctaantnnnnnagggcngt

SEQ ID NO: 9 - protein, 330 aa, synthetic construct
  REGION 1..330: note = Description of Artificial Sequence: Synthetic polypeptide
  MOD_RES 4: note = Any amino acid
  MOD_RES 296: note = Any amino acid
  MOD_RES 301: note = Any amino acid
  MOD_RES 303..305: note = Any amino acid
  MOD_RES 307: note = Any amino acid
  MOD_RES 315..317: note = Any amino acid
  MOD_RES 321: note = Any amino acid
  MOD_RES 324: note = Any amino acid
  MOD_RES 326..328: note = Any amino acid
  MOD_RES 330: note = Any amino acid
ILFXETVIMKYLLPTAAAGLLLLAAQPAMAQVQLQESGGGVVQPGRSLRLSCAASGFTFSTSGMHWVRQAPGKGLEWVAFILHDGSDKYYADSVKGRFTISRDNSKNTLYLQMNSLRAEDTAIYYCAKSQRELLGAEYLQNWGQGTLVTVSSGGGGSGGGGSGGGGSQSALTQPASVSGSPGQSITISCTGTSSDVGGYKYVSWYQQHPGKAPKVMIYDVSNRPSGVSNRFSGSKSGNTASLTISGLQAEDEADYYCSSYTSSSTLVFGGGTKVTVLGAAAEQKLISEEDLNGAAXTVESXLXXXIXKIHLLTSXXXTKLXIVXLXXXGX

SEQ ID NO: 10 - DNA, 1033 bp, synthetic construct
  misc_feature 1..1033: note = Description of Artificial Sequence: Synthetic polynucleotide
  modified_base 4: mod_base = OTHER; note = a, c, t, g, unknown or other
  modified_base 8: mod_base = OTHER; note = a, c, t, g, unknown or other
  modified_base 13..15: mod_base = OTHER; note = a, c, t, g, unknown or other
  modified_base 876: mod_base = OTHER; note = a, c, t, g, unknown or other
  modified_base 895: mod_base = OTHER; note = a, c, t, g, unknown or other
  modified_base 900..901: mod_base = OTHER; note = a, c, t, g, unknown or other
  modified_base 914: mod_base = OTHER; note = a, c, t, g, unknown or other
  modified_base 917: mod_base = OTHER; note = a, c, t, g, unknown or other
  modified_base 921..922: mod_base = OTHER; note = a, c, t, g, unknown or other
  modified_base 926..928: mod_base = OTHER; note = a, c, t, g, unknown or other
  modified_base 934: mod_base = OTHER; note = a, c, t, g, unknown or other
  modified_base 939: mod_base = OTHER; note = a, c, t, g, unknown or other
  modified_base 951..953: mod_base = OTHER; note = a, c, t, g, unknown or other
  modified_base 958: mod_base = OTHER; note = a, c, t, g, unknown or other
  modified_base 965..968: mod_base = OTHER; note = a, c, t, g, unknown or other
  modified_base 970..975: mod_base = OTHER; note = a, c, t, g, unknown or other
  modified_base 985..986: mod_base = OTHER; note = a, c, t, g, unknown or other
  modified_base 989..990: mod_base = OTHER; note = a, c, t, g, unknown or other
  modified_base 992: mod_base = OTHER; note = a, c, t, g, unknown or other
  modified_base 996..997: mod_base = OTHER; note = a, c, t, g, unknown or other
  modified_base 1002: mod_base = OTHER; note = a, c, t, g, unknown or other
  modified_base 1004..1007: mod_base = OTHER; note = a, c, t, g, unknown or other
  modified_base 1012..1017: mod_base = OTHER; note = a, c, t, g, unknown or other
  modified_base 1021: mod_base = OTHER; note = a, c, t, g, unknown or other
  modified_base 1023..1025: mod_base = OTHER; note = a, c, t, g, unknown or other
  modified_base 1027: mod_base = OTHER; note = a, c, t, g, unknown or other
  modified_base 1029..1032: mod_base = OTHER; note = a, c, t, g, unknown or other
  source 1..1033: mol_type = other DNA
gcanttcnatttnnngagacagtcataatgaaatacctattgcctacggcagccgctggattgttattactcgcggcccagccggccatggcccaggtgcagctggtggagtctgggggaggcttggtacagcctggggggtccctgagactctcctgtgcagcctctggattcacctttagcagctatgccatgagctgggtccgccaggctccagggaaggggctggagtgggtctcagctattagtggtagtggtggtagcacatactacgcagactccgtgaagggccggttcaccatctccagagacaattccaagaacacgctgtatctgcaaatgaacagcctgagagccgaggacacggctgtatattactgtgcaagaggtggcgattatggctcaggggactactggggccagggaaccctggtcaccgtctcctcaggtggaggcggttcaggcggaggtggctctggcggtggcggatcgaattttatgctgactcaggaccctgctgtgtctgtggccttgggacagacagtcagaatcacatgccaaggagacagcctcagaagctattatgcaagttggtaccagcagaagccaggacaggcccctctccttgtcatctatggtaaaaacatccggccctcagggatcccagaccgattctctggctccagctcaggaaactcagcttccttgaccatcactggggctcaggcggaagatgaggctgactattactgtcactcccgggacagcagtggtacccatctaagggtattcggcggagggaccaaggtcaccgtcctaggtgcggccgcagaacaaaaactcatctcagaagaggatctgaatggggccgcatanactgttgaaagttgtttancaaannctcatacagaaanttnattnnctannntctggnaagangacaaaactttnnntcgtnacgctannnntnnnnnntgtctgtganngcnncnggcnntgtgntnnnnactgnnnnnnaaantnnngntnnnng

SEQ ID NO: 11 - protein, 327 aa, synthetic construct
  REGION 1..327: note = Description of Artificial Sequence: Synthetic polypeptide
  MOD_RES 2..3: note = Any amino acid
  MOD_RES 5: note = Any amino acid
  MOD_RES 292: note = Any amino acid
  MOD_RES 299..301: note = Any amino acid
  MOD_RES 305..310: note = Any amino acid
  MOD_RES 312..313: note = Any amino acid
  MOD_RES 317..318: note = Any amino acid
  MOD_RES 320: note = Any amino acid
  MOD_RES 322..325: note = Any amino acid
AXXFXETVIMKYLLPTAAAGLLLLAAQPAMAQVQLVESGGGLVQPGGSLRLSCAASGFTFSSYAMSWVRQAPGKGLEWVSAISGSGGSTYYADSVKGRFTISRDNSKNTLYLQMNSLRAEDTAVYYCARGGDYGSGDYWGQGTLVTVSSGGGGSGGGGSGGGGSNFMLTQDPAVSVALGQTVRITCQGDSLRSYYASWYQQKPGQAPLLVIYGKNIRPSGIPDRFSGSSSGNSASLTITGAQAEDEADYYCHSRDSSGTHLRVFGGGTKVTVLGAAAEQKLISEEDLNGAAXTVESCLXXXHTEXXXXXXWXXDKTXXRXAXXXXCL

SEQ ID NO: 12 - DNA, 994 bp, synthetic construct
  misc_feature 1..994: note = Description of Artificial Sequence: Synthetic polynucleotide
  modified_base 3..5: mod_base = OTHER; note = a, c, t, g, unknown or other
  modified_base 876: mod_base = OTHER; note = a, c, t, g, unknown or other
  modified_base 895: mod_base = OTHER; note = a, c, t, g, unknown or other
  modified_base 905: mod_base = OTHER; note = a, c, t, g, unknown or other
  modified_base 908..910: mod_base = OTHER; note = a, c, t, g, unknown or other
  modified_base 927: mod_base = OTHER; note = a, c, t, g, unknown or other
  modified_base 952..953: mod_base = OTHER; note = a, c, t, g, unknown or other
  modified_base 971..972: mod_base = OTHER; note = a, c, t, g, unknown or other
  modified_base 978: mod_base = OTHER; note = a, c, t, g, unknown or other
  modified_base 982..983: mod_base = OTHER; note = a, c, t, g, unknown or other
  modified_base 985: mod_base = OTHER; note = a, c, t, g, unknown or other
  modified_base 987: mod_base = OTHER; note = a, c, t, g, unknown or other
  modified_base 993: mod_base = OTHER; note = a, c, t, g, unknown or other
  source 1..994: mol_type = other DNA
gcnnntctatttaaggagacagtcataatgaaatacctattgcctacggcagccgctggattgttattactcgcggcccagccggccatggcccaggtgcagctggtggcgtctggaggagacttgatccagcctggggggtccctgagactctcctgtgcagcctctggattcacctttaataactattggatgacctgggtccgccaggctccagggaaggggctggagtgggtggccaacataaagcaagatggaggtgagaaatactatgtggactctgtgaagggccgattcaccatctccagagacaacgccaagacctcactgtatctgcaaatgaacagcctgagagccgaggacacggccgtgtattattgtgcgaaagagtcgtatagcactggctggtttgaccactggggccagggaaccctggtcaccgtctcctcaggtggaggcggttcaggcggaggtggctctggcggtggcggatcgaattttatgctgactcaggaccctgctgtgtctgtggccttgggacagacagtcaggataacatgtcaaggtgacagcctcagaaaatattatacaagttggtaccaacagaagccaggacaggcccctctacttgtcatgtatgcgaaaaataaccggccctcagggatcccagaccgattctctggctccagctcaggaaacacagcttccttgaccatcactggggctcaggcggaagatgaggctgactattactgtgactcccgggacagcagtggtgaccattgggtgttcggcggagggaccaagctgaccgttctaggtgcggccgcagaacaaaaactcatctcagaagaggatctgaatggggccgcatanactgttgaaagttgtttancaaaacctcntannnaaaattcatttactaangtctggaaagacgacaaaactttanntcgttacgctaactatgnnggctgnctgnngnangctacng

SEQ ID NO: 13 - protein, 331 aa, synthetic construct
  REGION 1..331: note = Description of Artificial Sequence: Synthetic polypeptide
  MOD_RES 1..2: note = Any amino acid
  MOD_RES 292: note = Any amino acid
  MOD_RES 299: note = Any amino acid
  MOD_RES 302..304: note = Any amino acid
  MOD_RES 309: note = Any amino acid
  MOD_RES 318: note = Any amino acid
  MOD_RES 324: note = Any amino acid
  MOD_RES 326: note = Any amino acid
  MOD_RES 328..329: note = Any amino acid
  MOD_RES 331: note = Any amino acid
XXLFKETVIMKYLLPTAAAGLLLLAAQPAMAQVQLVASGGDLIQPGGSLRLSCAASGFTFNNYWMTWVRQAPGKGLEWVANIKQDGGEKYYVDSVKGRFTISRDNAKTSLYLQMNSLRAEDTAVYYCAKESYSTGWFDHWGQGTLVTVSSGGGGSGGGGSGGGGSNFMLTQDPAVSVALGQTVRITCQGDSLRKYYTSWYQQKPGQAPLLVMYAKNNRPSGIPDRFSGSSSGNTASLTITGAQAEDEADYYCDSRDSSGDHWVFGGGTKLTVLGAAAEQKLISEEDLNGAAXTVESCLXKPXXXNSFTXVWKDDKTLXRYANYXGXLXXAX

SEQ ID NO: 14 - DNA, 981 bp, synthetic construct
  misc_feature 1..981: note = Description of Artificial Sequence: Synthetic polynucleotide
  modified_base 2..5: mod_base = OTHER; note = a, c, t, g, unknown or other
  modified_base 8..10: mod_base = OTHER; note = a, c, t, g, unknown or other
  modified_base 865: mod_base = OTHER; note = a, c, t, g, unknown or other
  modified_base 870: mod_base = OTHER; note = a, c, t, g, unknown or other
  modified_base 884: mod_base = OTHER; note = a, c, t, g, unknown or other
  modified_base 894: mod_base = OTHER; note = a, c, t, g, unknown or other
  modified_base 931: mod_base = OTHER; note = a, c, t, g, unknown or other
  modified_base 941: mod_base = OTHER; note = a, c, t, g, unknown or other
  modified_base 950: mod_base = OTHER; note = a, c, t, g, unknown or other
  modified_base 959..961: mod_base = OTHER; note = a, c, t, g, unknown or other
  modified_base 964: mod_base = OTHER; note = a, c, t, g, unknown or other
  modified_base 971: mod_base = OTHER; note = a, c, t, g, unknown or other
  modified_base 973: mod_base = OTHER; note = a, c, t, g, unknown or other
  modified_base 975: mod_base = OTHER; note = a, c, t, g, unknown or other
  modified_base 978: mod_base = OTHER; note = a, c, t, g, unknown or other
  source 1..981: mol_type = other DNA
tnnnnttnnngagacagtcataatgaaatacctattgcctacggcagccgctggattgttattactcgcggcccagccggccatggcccgagtgcagctggtggagtctggggctgaggtgacgaagcctggggcctcagtaagggtctcctgcaaggcttctggatacaccttcagcagatatgatatcaactgggtgcgacaggcctctggacaagggcttgagtggatgggatggatcaaccctaacagtggtaacacaggctatgcacagaagttccagggcagagtcaccatgaccaggaatatttccataaccacggcctacatggagctgagcagcctgagatctgaggacacggccgtatattactgtgcgagaggccttccggagttcgacccctggggccagggaaccctggtcaccgtctcctcaggtggaggcggttcaggcggaggtggctctggcggtggcggatcgcacgttatactgactcaggaccctgctgtgtctgtggccttgggacagacagtcaggatcacatgccaaggagacagcctcagaagctattatgcaagctggtaccagcagaagccaggacaggcccctgtacttgtcatctatggtaaaaacaaccggccctcagggatcccagaccgattctctggctccagctcaggaaacacagcttccttgaccatcactggggctcaggcggaagatgaggctgacttttactgtaattcccgggacagcagtggcacccatctagaggtgttcggcggagggaccaaggtcaccgtcctaggtgcggccgcagaacaaaaactcatctcagaagaggatctgaatggggccgcatanactgntgaaagttgtttancaaaacctcntacagaaaattcatttactaacgtctggaaagacganaaaactttanatcgttacnctaactatnnnggntgtctgngnantgntac

SEQ ID NO: 15 - protein, 327 aa, synthetic construct
  REGION 1..327: note = Description of Artificial Sequence: Synthetic polypeptide
  MOD_RES 2..4: note = Any amino acid
  MOD_RES 289: note = Any amino acid
  MOD_RES 291: note = Any amino acid
  MOD_RES 296: note = Any amino acid
  MOD_RES 299: note = Any amino acid
  MOD_RES 311: note = Any amino acid
  MOD_RES 315: note = Any amino acid
  MOD_RES 318: note = Any amino acid
  MOD_RES 321..322: note = Any amino acid
  MOD_RES 325..327: note = Any amino acid
AXXXETVIMKYLLPTAAAGLLLLAAQPAMARVQLVESGAEVTKPGASVRVSCKASGYTFSRYDINWVRQASGQGLEWMGWINPNSGNTGYAQKFQGRVTMTRNISITTAYMELSSLRSEDTAVYYCARGLPEFDPWGQGTLVTVSSGGGGSGGGGSGGGGSHVILTQDPAVSVALGQTVRITCQGDSLRSYYASWYQQKPGQAPVLVIYGKNNRPSGIPDRFSGSSSGNTASLTITGAQAEDEADFYCNSRDSSGTHLEVFGGGTKVTVLGAAAEQKLISEEDLNGAAXTXESCLXKPXTENSFTNVWKDXKTLXRYXNYXXCLXXX

SEQ ID NO: 16 - DNA, 1041 bp, synthetic construct
  misc_feature 1..1041: note = Description of Artificial Sequence: Synthetic polynucleotide
  modified_base 2: mod_base = OTHER; note = a, c, t, g, unknown or other
  modified_base 11..13: mod_base = OTHER; note = a, c, t, g, unknown or other
  modified_base 706: mod_base = OTHER; note = a, c, t, g, unknown or other
  modified_base 746: mod_base = OTHER; note = a, c, t, g, unknown or other
  modified_base 748: mod_base = OTHER; note = a, c, t, g, unknown or other
  modified_base 771..773: mod_base = OTHER; note = a, c, t, g, unknown or other
  modified_base 796: mod_base = OTHER; note = a, c, t, g, unknown or other
  modified_base 803: mod_base = OTHER; note = a, c, t, g, unknown or other
  modified_base 815: mod_base = OTHER; note = a, c, t, g, unknown or other
  modified_base 833: mod_base = OTHER; note = a, c, t, g, unknown or other
  modified_base 851: mod_base = OTHER; note = a, c, t, g, unknown or other
  modified_base 855: mod_base = OTHER; note = a, c, t, g, unknown or other
  modified_base 857: mod_base = OTHER; note = a, c, t, g, unknown or other
  modified_base 859..860: mod_base = OTHER; note = a, c, t, g, unknown or other
  modified_base 862: mod_base = OTHER; note = a, c, t, g, unknown or other
  modified_base 875: mod_base = OTHER; note = a, c, t, g, unknown or other
  modified_base 878: mod_base = OTHER; note = a, c, t, g, unknown or other
  modified_base 883: mod_base = OTHER; note = a, c, t, g, unknown or other
  modified_base 900: mod_base = OTHER; note = a, c, t, g, unknown or other
  modified_base 913: mod_base = OTHER; note = a, c, t, g, unknown or other
  modified_base 917: mod_base = OTHER; note = a, c, t, g, unknown or other
  modified_base 925: mod_base = OTHER; note = a, c, t, g, unknown or other
  modified_base 928..931: mod_base = OTHER; note = a, c, t, g, unknown or other
  modified_base 933: mod_base = OTHER; note = a, c, t, g, unknown or other
  modified_base 935..936: mod_base = OTHER; note = a, c, t, g, unknown or other
  modified_base 944: mod_base = OTHER; note = a, c, t, g, unknown or other
  modified_base 946: mod_base = OTHER; note = a, c, t, g, unknown or other
  modified_base 948: mod_base = OTHER; note = a, c, t, g, unknown or other
  modified_base 950..952: mod_base = OTHER; note = a, c, t, g, unknown or other
  modified_base 954..955: mod_base = OTHER; note = a, c, t, g, unknown or other
  modified_base 957..958: mod_base = OTHER; note = a, c, t, g, unknown or other
  modified_base 966: mod_base = OTHER; note = a, c, t, g, unknown or other
  modified_base 969: mod_base = OTHER; note = a, c, t, g, unknown or other
  modified_base 971: mod_base = OTHER; note = a, c, t, g, unknown or other
  modified_base 973: mod_base = OTHER; note = a, c, t, g, unknown or other
  modified_base 977..980: mod_base = OTHER; note = a, c, t, g, unknown or other
  modified_base 983: mod_base = OTHER; note = a, c, t, g, unknown or other
  modified_base 985..988: mod_base = OTHER; note = a, c, t, g, unknown or other
  modified_base 990..992: mod_base = OTHER; note = a, c, t, g, unknown or other
  modified_base 994: mod_base = OTHER; note = a, c, t, g, unknown or other
  modified_base 996: mod_base = OTHER; note = a, c, t, g, unknown or other
  modified_base 998..999: mod_base = OTHER; note = a, c, t, g, unknown or other
  modified_base 1001..1011: mod_base = OTHER; note = a, c, t, g, unknown or other
  modified_base 1013: mod_base = OTHER; note = a, c, t, g, unknown or other
  modified_base 1015..1017: mod_base = OTHER; note = a, c, t, g, unknown or other
  modified_base 1020: mod_base = OTHER; note = a, c, t, g, unknown or other
  modified_base 1022..1027: mod_base = OTHER; note = a, c, t, g, unknown or other
  modified_base 1029..1034: mod_base = OTHER; note = a, c, t, g, unknown or other
  modified_base 1036: mod_base = OTHER; note = a, c, t, g, unknown or other
  modified_base 1040: mod_base = OTHER; note = a, c, t, g, unknown or other
  source 1..1041: mol_type = other DNA
anttctatttnnngagacagtcataatgaaatacctattgcctacggcagccgctggattgttattactcgcggcccagccggccatggcccaggtacagctgcaggagtctgggggaggcttggtccagcctgggaggtccctgagactctcctgtgcagcctctggattcaccttcagtaactttggcatgcactgggtctgccaggctccaggcaaggggctggagtgggtggcaattatttcatatgatgcaagtagtgaatactatgcagactccgtgaagggccgattcaccatctccagagacaattccaggaacactctttatctgcaaatgaacagcctgagacctgaggacacggctgtatattactgtgcgaagaaggacggtcggagtgggagctactactactttgactactggggccagggaaccctggtcaccgtctcctcaggtggaggcggttcaggcggaggtggctctggcggtggcggatcggatgttgtgatgactcagtctccatcctccctgtctgcatctgtaggagacagagtcaccatcacttgccgggcgagtcaagattttaggaattggttagcctggtatcaggtgaaaccaggaaaagcccccaagcccctgatctatggtgcatccactttgcaaaatggggtcccatccaggttcagcggcagtgggtctganacagatttctctctcactatcagcagcctgcagcctgagnantttgcaacttacttttgtcaacnnntcacagtttccctcccactttcncggaggnacacgactgganatcaaacgtgcggccgcncatcatcatcaccatcangggncncnnanaaaactcatctcnaanagganctgaatgggccgcatanactgtgaagttgnttancaaactcntannnnantnntttactangncngnnnannannaacttaantcntncnctannnngangnnnncnnngnangnnannnnnnnnnnngntnnnacngnnnnnnannnnnngntacng

SEQ ID NO: 17 - protein, 301 aa, synthetic construct
  REGION 1..301: note = Description of Artificial Sequence: Synthetic polypeptide
  MOD_RES 1: note = Any amino acid
  MOD_RES 4: note = Any amino acid
  MOD_RES 235: note = Any amino acid
  MOD_RES 249: note = Any amino acid
  MOD_RES 257..258: note = Any amino acid
  MOD_RES 265: note = Any amino acid
  MOD_RES 268: note = Any amino acid
  MOD_RES 272: note = Any amino acid
  MOD_RES 278: note = Any amino acid
  MOD_RES 284..287: note = Any amino acid
  MOD_RES 292..294: note = Any amino acid
  MOD_RES 300: note = Any amino acid
XLFXETVIMKYLLPTAAAGLLLLAAQPAMAQVQLQESGGGLVQPGRSLRLSCAASGFTFSNFGMHWVCQAPGKGLEWVAIISYDASSEYYADSVKGRFTISRDNSRNTLYLQMNSLRPEDTAVYYCAKKDGRSGSYYYFDYWGQGTLVTVSSGGGGSGGGGSGGGGSDVVMTQSPSSLSASVGDRVTITCRASQDFRNWLAWYQVKPGKAPKPLIYGASTLQNGVPSRFSGSGSXTDFSLTISSLQPEXFATYFCQXXTVSLPLXRRXTTGXQTCGRXSSSPSXXXXKTHLXXXLNGPHXL

SEQ ID NO: 18 - DNA, 989 bp, synthetic construct
  misc_feature 1..989: note = Description of Artificial Sequence: Synthetic polynucleotide
  modified_base 2..5: mod_base = OTHER; note = a, c, t, g, unknown or other
  modified_base 8: mod_base = OTHER; note = a, c, t, g, unknown or other
  modified_base 13..15: mod_base = OTHER; note = a, c, t, g, unknown or other
  modified_base 691: mod_base = OTHER; note = a, c, t, g, unknown or other
  modified_base 727: mod_base = OTHER; note = a, c, t, g, unknown or other
  modified_base 877: mod_base = OTHER; note = a, c, t, g, unknown or other
  modified_base 896: mod_base = OTHER; note = a, c, t, g, unknown or other
  modified_base 898: mod_base = OTHER; note = a, c, t, g, unknown or other
  modified_base 910..911: mod_base = OTHER; note = a, c, t, g, unknown or other
  modified_base 935: mod_base = OTHER; note = a, c, t, g, unknown or other
  modified_base 938: mod_base = OTHER; note = a, c, t, g, unknown or other
  modified_base 941: mod_base = OTHER; note = a, c, t, g, unknown or other
  modified_base 952: mod_base = OTHER; note = a, c, t, g, unknown or other
  modified_base 980: mod_base = OTHER; note = a, c, t, g, unknown or other
  modified_base 982: mod_base = OTHER; note = a, c, t, g, unknown or other
  modified_base 984: mod_base = OTHER; note = a, c, t, g, unknown or other
  source 1..989: mol_type = other DNA
gnnnntcnatttnnngagacagtcataatgaaatacctattgcctacggcagccgctggattgttattactcgcggcccagccggccatggcccaggtgcagctgcaggagtctgggggagacgtggtccagcctgggaggtccctgagactctcctgtgcagcctctggattcaccttcagtagctatggcatgcactgggtccgccaggctccaggcaaggggctggagtgggtggcagttatatcatatgatgaaagtaataaatactatgcagactccgtgaagggccgattcaccatctccagagacaattccaagaacacactgtttctgcaaatgaacagcctgagagctgaggacacggctgtgtattactgtgcgaaaggacctgtcctaactggggagtttgactattggggccgtagaaccctggtcaccgtctcctcaggtggaggcggttcaggcggaggtggctctggcggtggcggatcgtctgagctgactcaggaccctgctgtgtctgtggccttgggacagacagtcaggatcacatgccaaggagacagcctcaaaagctactatgcaagttggtaccagcagaagccaggacaggcccctgtacttgtcatctatggtgaaaacagccggccctccgggatcccagaccgattctctggttccagctcangaaacacagcttccttgaccatcactgggggctcangcggaagatgaagctgactattattgtaactcccgggacaacagtggtacccatcttgaggtattcggcggagggaccaagctgaccgtcctaggtgcggccgcagaacaaaaactcatctcagaagaggatctgaatggggccgcatanactgttgaaagttgtttancnaaacctcatacnnaaaattcatttactaacgtctggnaanacnacaaactttanatcgttacgctaactatgagggctgtcngngnaatgc

SEQ ID NO: 19 - protein, 245 aa, synthetic construct
  REGION 1..245: note = Description of Artificial Sequence: Synthetic polypeptide
  MOD_RES 1..3: note = Any amino acid
  MOD_RES 5: note = Any amino acid
  MOD_RES 231: note = Any amino acid
  MOD_RES 243: note = Any amino acid
XXXFXETVIMKYLLPTAAAGLLLLAAQPAMAQVQLQESGGDVVQPGRSLRLSCAASGFTFSSYGMHWVRQAPGKGLEWVAVISYDESNKYYADSVKGRFTISRDNSKNTLFLQMNSLRAEDTAVYYCAKGPVLTGEFDYWGRRTLVTVSSGGGGSGGGGSGGGGSSELTQDPAVSVALGQTVRITCQGDSLKSYYASWYQQKPGQAPVLVIYGENSRPSGIPDRFSGSSSXNTASLTITGGSXGR

SEQ ID NO: 20 - DNA, 892 bp, synthetic construct
  misc_feature 1..892: note = Description of Artificial Sequence: Synthetic polynucleotide
  source 1..892: mol_type = other DNA
gagacagtcataatgaaatacctattgcctacggcagccgctggattgttattactcgcggcccagccggccatggcccaggtacagctgcaggagtctgggggaggcttggtacagcctggggggtccctgagactctcctgtgcagcctctggattcacctttagcagctatgccatgagctgggtccgccaggctccagggaaggggctggagtgggtctcagctattagtggtagtggtggtagcacatactacgcagactccgtgaagggccgattcaccatctccagagacaattccaagaacacgctgtatctgcaaatgaacagcctgagagctgaggacacggctgtgtattactgtgcgaagagctatggttcagttaaaataagctgctttgactactggggccagagcaccctggtcaccgtctcctcaggtggaggcggttcaggcggaggtggctctggcggtggcggatcggaaattgtgctgacgcagtctccagactccctggctgtgtctctgggcgagagggccaccatcaactgcaagtccagccagagtgttctttacaactccaacaataagaactacttagcttggtaccagcagaaaccaggacagtctcctgagttgctcatttactgggcatcaacccgggaatccggggtccctgaccgattcagtggcagcgggtctgggacagaattcactcttaccatcagcagcctgcaggctgaggatgtggcagtttattactgtcagcaattttatagtactcctccgacttttggccaggggaccaagctggagatcaaacgtgcggccgcacatcatcatcaccatcacggggccgcagaacaaaaactcatctcagaagaggatc

SEQ ID NO: 21 - DNA, 977 bp, synthetic construct
  misc_feature 1..977: note = Description of Artificial Sequence: Synthetic polynucleotide
  modified_base 3..5: mod_base = OTHER; note = a, c, t, g, unknown or other
  modified_base 13..15: mod_base = OTHER; note = a, c, t, g, unknown or other
  modified_base 707: mod_base = OTHER; note = a, c, t, g, unknown or other
  modified_base 747: mod_base = OTHER; note = a, c, t, g, unknown or other
  modified_base 749: mod_base = OTHER; note = a, c, t, g, unknown or other
  modified_base 772: mod_base = OTHER; note = a, c, t, g, unknown or other
  modified_base 775: mod_base = OTHER; note = a, c, t, g, unknown or other
  modified_base 799..800: mod_base = OTHER; note = a, c, t, g, unknown or other
  modified_base 808: mod_base = OTHER; note = a, c, t, g, unknown or other
  modified_base 830: mod_base = OTHER; note = a, c, t, g, unknown or other
  modified_base 836..837: mod_base = OTHER; note = a, c, t, g, unknown or other
  modified_base 852..853: mod_base = OTHER; note = a, c, t, g, unknown or other
  modified_base 855..858: mod_base = OTHER; note = a, c, t, g, unknown or other
  modified_base 872: mod_base = OTHER; note = a, c, t, g, unknown or other
  modified_base 877: mod_base = OTHER; note = a, c, t, g, unknown or other
  modified_base 882: mod_base = OTHER; note = a, c, t, g, unknown or other
  modified_base 890..891: mod_base = OTHER; note = a, c, t, g, unknown or other
  modified_base 895: mod_base = OTHER; note = a, c, t, g, unknown or other
  modified_base 901..902: mod_base = OTHER; note = a, c, t, g, unknown or other
  modified_base 904: mod_base = OTHER; note = a, c, t, g, unknown or other
  modified_base 908..909: mod_base = OTHER; note = a, c, t, g, unknown or other
  modified_base 920: mod_base = OTHER; note = a, c, t, g, unknown or other
  modified_base 928: mod_base = OTHER; note = a, c, t, g, unknown or other
  modified_base 933: mod_base = OTHER; note = a, c, t, g, unknown or other
  modified_base 935..936: mod_base = OTHER; note = a, c, t, g, unknown or other
  modified_base 938..939: mod_base = OTHER; note = a, c, t, g, unknown or other
  modified_base 942: mod_base = OTHER; note = a, c, t, g, unknown or other
  modified_base 947: mod_base = OTHER; note = a, c, t, g, unknown or other
  modified_base 950: mod_base = OTHER; note = a, c, t, g, unknown or other
  modified_base 953: mod_base = OTHER; note = a, c, t, g, unknown or other
  modified_base 955: mod_base = OTHER; note = a, c, t, g, unknown or other
  modified_base 957: mod_base = OTHER; note = a, c, t, g, unknown or other
  modified_base 959: mod_base = OTHER; note = a, c, t, g, unknown or other
  modified_base 964..965: mod_base = OTHER; note = a, c, t, g, unknown or other
  modified_base 967..968: mod_base = OTHER; note = a, c, t, g, unknown or other
  modified_base 970: mod_base = OTHER; note = a, c, t, g, unknown or other
  modified_base 972..976: mod_base = OTHER; note = a, c, t, g, unknown or other
  source 1..977: mol_type = other DNA
gcnnntctatttnnngagacagtcataatgaaatacctattgcctacggcagccgctggattgttattactcgcggcccagccggccatggcccaggtgcagctgtggagtctgggggaggcgtggtccagcctgggaggtccctgagactctcctgtgcagcctctggattcaccttcagtaactttggcatgcactgggtctgccaggctccaggcaaggggctggagtgggtggcaattatttcatatgatgcaagtagtgaatactatgcagactccgtgaagggccgattcaccatctccagagacaattccaggaacactctttatctgcaaatgaacagcctgagacctgaggacacggctgtatattactgtgcgaagaaggacggtcggagtgggagctactactactttgactactggggccagggaaccctggtcaccgtctcctcaggtggaggcggttcaggcggaggtggctctggcggtggcggatcggatgttgtgatgactcagtctccatcctccctgtctgcatctgtaggagacagagtcaccatcacttgccgggcgagtcaagattttaggaattggttagcctggtatcaggtgaaaccaggaaaagcccccaagcccctgatctatggtgcatccactttgcaaaatggggtcccatccaggttcagcggcagtgggtctganacagatttctctctcactatcagcagcctgcagcctgagnantttgcaacttacttttgtcaacnggntcacagtttccctcccactttcgnnggaggganacgactggagattaaacgtgcngccgcnnacaaaactcatctcnnannnntctgaatggggccncatanactgntgaaagtnnttancaaacnncntacnnaaaattcattnctacgtcnggaanannannaantttanatngtncncnantatgnngnngncnnnnna

SEQ ID NO: 22 - DNA, 13 bp, synthetic construct
  misc_feature 1..13: note = Description of Artificial Sequence: Synthetic oligonucleotide
  source 1..13: mol_type = other DNA
ggcccagccggcc

SEQ ID NO: 23 - DNA, 109 bp, synthetic construct
  misc_feature 1..109: note = Description of Artificial Sequence: Synthetic polynucleotide
  source 1..109: mol_type = other DNA
ggcccagccggccatggcccaggtgcagctggtgcagtctggggctgaggtgaagaagcctggggcctcagtgaaggtctcctgcaaggcttctggttacacctttacc

SEQ ID NO: 24 - DNA, 109 bp, synthetic construct
  misc_feature 1..109: note = Description of Artificial Sequence: Synthetic polynucleotide
  source 1..109: mol_type = other DNA
ggcccagccggccatggcccaggtgcagctggtgcagtctgggggaggcgtggtccagcctgggaggtccctgagactctcctgtgcagcctctggattcaccttcagt

SEQ ID NO: 25 - DNA, 109 bp, synthetic construct
  misc_feature 1..109: note = Description of Artificial Sequence: Synthetic polynucleotide
  source 1..109: mol_type = other DNA
ggcccagccggccatggcccaggtacagctgcagcagtcaggctcaggactggtgaagccttcacagaccctgtccctcacctgctctgtctctggtgactccatctcc

SEQ ID NO: 26 - DNA, 109 bp, synthetic construct
  misc_feature 1..109: note = Description of Artificial Sequence: Synthetic polynucleotide
  source 1..109: mol_type = other DNA
ggcccagccggccatggcccaggtgcagctgcaggagtcggggccaggactggtgaagccttcggagaccctgtccctcgtctgcactgtctctggtggctccctcagt

SEQ ID NO: 27 - DNA, 109 bp, synthetic construct
  misc_feature 1..109: note = Description of Artificial Sequence: Synthetic polynucleotide
  source 1..109: mol_type = other DNA
ggcccagccggccatggcccaggtgcagctggtgcagtctggagcagaggtgaaaaagcccgggcagtctctgatgatctcctgtcagggttctggatacagctttagc

SEQ ID NO: 28 - DNA, 109 bp, synthetic construct
  misc_feature 1..109: note = Description of Artificial Sequence: Synthetic polynucleotide
  source 1..109: mol_type = other DNA
ggcccagccggccatggcccaggtgcagctggtgcagtctggggcagaggtgaaaaagcccgggcagtctctgaggatctcctgtaagggtgctggatacagctttagc

SEQ ID NO: 29 - DNA, 108 bp, synthetic construct
  misc_feature 1..108: note = Description of Artificial Sequence: Synthetic polynucleotide
  source 1..108: mol_type = other DNA
ggcccagccggccatggcccaggtgcagctgcaggagtcgggggaggcgtggtccagcctgggaggtccctgagactctcctgtgcagcgtctggattcaccttcagt

SEQ ID NO: 30 - DNA, 108 bp, synthetic construct
  misc_feature 1..108: note = Description of Artificial Sequence: Synthetic polynucleotide
  source 1..108: mol_type = other DNA
ggcccagccggccatggccaggtgcagctggtggagtctgggggaggcttggtacagcctggggggtccctgagactctcctgtgcagcctctggattcacctttagc

SEQ ID NO: 31 - DNA, 108 bp, synthetic construct
  misc_feature 1..108: note = Description of Artificial Sequence: Synthetic polynucleotide
  source 1..108: mol_type = other DNA
ggcccagccggccatggcccaggtgcagctgtggagtctgggggaggcgtggtccagcctgggaggtccctgagactctcctgtgcagcctctggattcaccttcagt

SEQ ID NO: 32 - DNA, 108 bp, synthetic construct
  misc_feature 1..108: note = Description of Artificial Sequence: Synthetic polynucleotide
  source 1..108: mol_type = other DNA
ggcccagccggccatggcccaggtgcagctggtgcgtctggaggagacttgatccagcctggggggtccctgagactctcctgtgcagcctctggattcacctttaat

SEQ ID NO: 33 - DNA, 108 bp, synthetic construct
  misc_feature 1..108: note = Description of Artificial Sequence: Synthetic polynucleotide
  source 1..108: mol_type = other DNA
ggcccagccggccatggcccaggtgcagctgcaggagtcgggggagacgtggtccagcctgggaggtccctgagactctcctgtgcagcctctggattcaccttcagt

SEQ ID NO: 34 - DNA, 108 bp, synthetic construct
  misc_feature 1..108: note = Description of Artificial Sequence: Synthetic polynucleotide
  source 1..108: mol_type = other DNA
ggcccagccggccatggccgagtgcagctggtggagtctggggctgaggtgacgaagcctggggcctcagtaagggtctcctgcaaggcttctggatacaccttcagc

SEQ ID NO: 35 - DNA, 51 bp, synthetic construct
  misc_feature 1..51: note = Description of Artificial Sequence: Synthetic primer
  source 1..51: mol_type = other DNA
atatatccatggcccaggtgcagctgcaggagtctgggggaggcgtggtcc

SEQ ID NO: 36 - DNA, 51 bp, synthetic construct
  misc_feature 1..51: note = Description of Artificial Sequence: Synthetic primer
  source 1..51: mol_type = other DNA
atatatccatggcccaggtgcagctggtggagtctgggggaggcttggtac

SEQ ID NO: 37 - DNA, 48 bp, synthetic construct
  misc_feature 1..48: note = Description of Artificial Sequence: Synthetic primer
  source 1..48: mol_type = other DNA
gccggccatggcccaggtacagctgcaggagtctgggggaggcttggt

SEQ ID NO: 38 - DNA, 45 bp, synthetic construct
  misc_feature 1..45: note = Description of Artificial Sequence: Synthetic primer
  source 1..45: mol_type = other DNA
cccgtgatggtgatgatgatgtgcggccgcacgtttgatctccag

SEQ ID NO: 39 - protein, 6 aa, synthetic construct
  REGION 1..6: note = Description of Artificial Sequence: Synthetic peptide
VQIINK

SEQ ID NO: 40 - protein, 6 aa, synthetic construct
  REGION 1..6: note = Description of Artificial Sequence: Synthetic peptide
VQIVYK

SEQ ID NO: 41 - protein, 201 aa, synthetic construct
  REGION 1..201: note = Description of Artificial Sequence: Synthetic polypeptide
  REGION 1..100: note = misc_feature - This region may encompass 3-100 "Gly" residues
  REGION 102..201: note = misc_feature - This region may encompass 3-100 "Gly" residues
GGGGGGGGGGGGGGGGGGGGGGGGGGGGGGGGGGGGGGGGGGGGGGGGGGGGGGGGGGGGGGGGGGGGGGGGGGGGGGGGGGGGGGGGGGGGGGGGGGGGPGGGGGGGGGGGGGGGGGGGGGGGGGGGGGGGGGGGGGGGGGGGGGGGGGGGGGGGGGGGGGGGGGGGGGGGGGGGGGGGGGGGGGGGGGGGGGGGGGGGG

SEQ ID NO: 42 - protein, 6 aa, synthetic construct
  REGION 1..6: note = Description of Artificial Sequence: Synthetic 6xHis tag
HHHHHH

SEQ ID NO: 43 - skipped

SEQ ID NO: 44 - protein, 45 aa, synthetic construct
  REGION 1..45: note = Description of Artificial Sequence: Synthetic polypeptide
  MOD_RES 2: note = Any amino acid
  MOD_RES 4: note = Any amino acid
  MOD_RES 6..10: note = Any amino acid
  MOD_RES 13..17: note = Any amino acid
  MOD_RES 20..22: note = Any amino acid
  MOD_RES 24..43: note = Any amino acid
  MOD_RES 45: note = Any amino acid
SXLXNXXXXXLLXXXXXNLXXXLXXXXXXXXXXXXXXXXXXXXYX

SEQ ID NO: 45-46 - skipped (2 entries)

SEQ ID NO: 47 - protein, 9 aa, synthetic construct
  REGION 1..9: note = Description of Artificial Sequence: Synthetic peptide
LPGQQWYPS

SEQ ID NO: 48 - protein, 32 aa, synthetic construct
  REGION 1..32: note = Description of Artificial Sequence: Synthetic polypeptide
  MOD_RES 31: note = Any amino acid
GIRRRDQADRPRCGRRTKTHLRRGSEWGRIXC

SEQ ID NO: 49 - protein, 13 aa, synthetic construct
  REGION 1..13: note = Description of Artificial Sequence: Synthetic peptide
  MOD_RES 4..5: note = Any amino acid
  MOD_RES 9: note = Any amino acid
KLFXXTSYXKFIY

SEQ ID NO: 50 - protein, 20 aa, synthetic construct
  REGION 1..20: note = Description of Artificial Sequence: Synthetic peptide
  MOD_RES 3..5: note = Any amino acid
  MOD_RES 9: note = Any amino acid
  MOD_RES 18..19: note = Any amino acid
RLXXXQTLXRYANYEGCXXN